European Patent Application EP 4 257 687 A1, published October 11, 2023. Title: Novel L-rhamnose isomerase. Applicant: NATIONAL UNIVERSITY CORPORATION KAGAWA UNIVERSITY. The sequence listing filed with the application follows.

SEQUENCE LISTING (2 sequences)

SEQ ID NO: 1 - protein, 419 aa, Enterobacter roggenkampii
MTTQLEQAWDLAKQRFAAVGVDVEEALRQLDRLPVSMHCWQGDDVAGFENPGGSLTGGIQATGNYPGKARNATELRADLELTLSLIPGPKRLNLHAIYLESDEPVARNEIKPEHFKNWVEWAKANKLGLDFNPSCFSHPLSADGFTLAHADDEIRQFWIDHVKASRRVSAYFGEQLGTPSVMNIWIPDGMKDITVDRLAPRQRLLAALDEAISEKLDPAHHIDAVESKLFGIGAESYTVGSNEFYMGYATSRQTALCLDAGHFHPTEVISDKISAAMLYVPRLLLHVSRPVRWDSDHVVLLDDETQAIASEIIRHDLFDRVHIGLDFFDASINRIAAWVIGTRNMKKALLRALLEPTAELKKLEANGDYTARLALLEEQKSLPWQAVWEMYCQRNDAPAGSQWLDNVRAYEEDVLSQRG

SEQ ID NO: 2 - DNA, 1260 bp, Enterobacter roggenkampii
atgaccactcaattagaacaagcctgggacctggctaaacagcgtttcgccgccgtcggcgtggatgtcgaagaggccctgcgccagctcgaccgtctgcccgtctctatgcactgctggcagggcgatgacgtcgccggtttcgagaacccgggcggttccctgacgggtggtattcaggccacgggtaattatccgggcaaagcgcgtaacgcgaccgagctgcgcgccgatctggagctgaccctgagcctgatcccggggccaaagcgcctgaacctgcacgcgatttacctcgagtccgacgagccggtggcgcgcaacgaaatcaaaccggagcattttaagaactgggtggagtgggcaaaagccaataagctgggcctggatttcaacccatcctgcttctcgcatccgctgagcgcggacggttttaccctcgcccacgcggacgatgaaatccgtcagttctggatcgaccacgtgaaggccagccgccgcgtgtctgcgtactttggcgagcagctcggcacaccgtcggtgatgaacatctggatcccggacggcatgaaggacatcaccgtcgaccgtcttgctccgcgccagcgcctgctggccgcgctggatgaggccatcagcgagaagctggacccggcgcaccacatcgacgccgtggagagcaagctgttcggcattggcgccgagagctacaccgtcggctcgaacgagttctacatggggtacgccaccagccgccagaccgcgctgtgcctggatgccggtcacttccatccgaccgaggtgatctccgacaaaatctccgctgccatgctctacgtgccgcgcctgctgctgcacgtcagccgtccggtgcgctgggacagcgaccacgtagtgctgctggatgacgaaacccaggcgattgcgagcgaaatcatccgccacgacctctttgaccgcgtccacatcggcctcgacttcttcgatgcctccatcaaccgcatcgcggcgtgggttatcggcacccgcaacatgaagaaagccctgctgcgcgccctgctggagccgactgccgaactgaaaaagctggaagcaaacggtgactacaccgcgcgtctggcgctgctggaagagcagaaatctctgccgtggcaggcggtgtgggagatgtactgccagcgtaacgacgccccggcgggcagccagtggctggacaacgtgcgggcgtatgaggaagacgtgttgagtcagcgcgggtaa